European Patent Specification EP 3 833 366 B1, published December 3, 2025. Title: MICROORGANISM MIXTURES, MOLECULES DERIVED THEREFROM, AND METHODS OF USE THEREOF. Applicant: B. G. NEGEV TECHNOLOGIES AND APPLICATIONS LTD., AT BEN-GURION UNIVERSITY. The sequence listing filed with the application follows.

SEQUENCE LISTING (8 sequences)

SEQ ID NO: 1 - DNA, 21 bp, Artificial Sequence
  Synthetic
ctggcggcattggtcaagccc

SEQ ID NO: 2 - DNA, 20 bp, Artificial Sequence
  Synthetic
acccggtgtgacaggcgcaa

SEQ ID NO: 3 - DNA, 21 bp, Artificial Sequence
  Synthetic
cgcagtattcagatgctggtg

SEQ ID NO: 4 - DNA, 21 bp, Artificial Sequence
  Synthetic
gacctctttcgcatcaggaca

SEQ ID NO: 5 - DNA, 21 bp, Artificial Sequence
  Synthetic
agcagtcaggtggtcttatgc

SEQ ID NO: 6 - DNA, 20 bp, Artificial Sequence
  Synthetic
cccgtctgagttcctcttgc

SEQ ID NO: 7 - DNA, 24 bp, Artificial Sequence
  Synthetic
accgggtacgatataaccaaagag

SEQ ID NO: 8 - DNA, 20 bp, Artificial Sequence
  Synthetic
gatggctggctttccagaag